European Patent Specification EP 3 419 651 B1, published October 25, 2023. Title: TARGETED THERAPEUTIC LYSOSOMAL ENZYME FUSION PROTEINS, ASSOCIATED FORMULATIONS AND USES THEREOF. Applicant: BIOMARIN PHARMACEUTICAL INC. The sequence listing filed with the application follows.

SEQUENCE LISTING (5 sequences)

SEQ ID NO: 1 - protein, 720 aa, Homo sapiens
  MISC_FEATURE: Naglu protein
DEAREAAAVRALVARLLGPGPAADFSVSVERALAAKPGLDTYSLGGGGAARVRVRGSTGVAAAAGLHRYLRDFCGCHVAWSGSQLRLPRPLPAVPGELTEATPNRYRYYQNVCTQSYSFVWWDWARWEREIDWMALNGINLALAWSGQEAIWQRVYLALGLTQAEINEFFTGPAFLAWGRMGNLHTWDGPLPPSWHIKQLYLQHRVLDQMRSFGMTPVLPAFAGHVPEAVTRVFPQVNVTKMGSWGHFNCSYSCSFLLAPEDPIFPIIGSLFLRELIKEFGTDHIYGADTFNEMQPPSSEPSYLAAATTAVYEAMTAVDTEAVWLLQGWLFQHQPQFWGPAQIRAVLGAVPRGRLLVLDLFAESQPVYTRTASFQGQPFIWCMLHNFGGNHGLFGALEAVNGGPEAARLFPNSTMVGTGMAPEGISQNEVVYSLMAELGWRKDPVPDLAAWVTSFAARRYGVSHPDAGAAWRLLLRSVYNCSGEACRGHNRSPLVRRPSLQMNTSIWYNRSDVFEAWRLLLTSAPSLATSPAFRYDLLDLTRQAVQELVSLYYEEARSAYLSKELASLLRAGGVLAYELLPALDEVLASDSRFLLGSWLEQARAAAVSEAEADFYEQNSRYQLTLWGPEGNILDYANKQLAGLVANYYTPRWRLFLEALVDSVAQGIPFQQHQFDKNVFQLEQAFVLSKQRYPSQPRGDTVDLAKKIFLKYYPRWVAGSW

SEQ ID NO: 2 - protein, 60 aa, Homo sapiens
  MISC_FEATURE: AA 8-67 of IGF-II
LCGGELVDTLQFVCGDRGFYFSRPASRVSRRSRGIVEECCFRSCDLALLETYCATPAKSE

SEQ ID NO: 3 - protein, 60 aa, Artificial Sequence
  Peptide Tag
LCGGELVDTLQFVCGDRGFYFSRPASRVSARSRGIVEECCFRSCDLALLETYCATPAKSE

SEQ ID NO: 4 - protein, 31 aa, Artificial Sequence
  Peptide Linker
GAPGGGSPAPAPTPAPAPTPAPAGGGPSGAP

SEQ ID NO: 5 - protein, 811 aa, Artificial Sequence
  Synthetic Polypeptide
  MISC_FEATURE: BMN001 therapeutic fusion protein
DEAREAAAVRALVARLLGPGPAADFSVSVERALAAKPGLDTYSLGGGGAARVRVRGSTGVAAAAGLHRYLRDFCGCHVAWSGSQLRLPRPLPAVPGELTEATPNRYRYYQNVCTQSYSFVWWDWARWEREIDWMALNGINLALAWSGQEAIWQRVYLALGLTQAEINEFFTGPAFLAWGRMGNLHTWDGPLPPSWHIKQLYLQHRVLDQMRSFGMTPVLPAFAGHVPEAVTRVFPQVNVTKMGSWGHFNCSYSCSFLLAPEDPIFPIIGSLFLRELIKEFGTDHIYGADTFNEMQPPSSEPSYLAAATTAVYEAMTAVDTEAVWLLQGWLFQHQPQFWGPAQIRAVLGAVPRGRLLVLDLFAESQPVYTRTASFQGQPFIWCMLHNFGGNHGLFGALEAVNGGPEAARLFPNSTMVGTGMAPEGISQNEVVYSLMAELGWRKDPVPDLAAWVTSFAARRYGVSHPDAGAAWRLLLRSVYNCSGEACRGHNRSPLVRRPSLQMNTSIWYNRSDVFEAWRLLLTSAPSLATSPAFRYDLLDLTRQAVQELVSLYYEEARSAYLSKELASLLRAGGVLAYELLPALDEVLASDSRFLLGSWLEQARAAAVSEAEADFYEQNSRYQLTLWGPEGNILDYANKQLAGLVANYYTPRWRLFLEALVDSVAQGIPFQQHQFDKNVFQLEQAFVLSKQRYPSQPRGDTVDLAKKIFLKYYPRWVAGSWGAPGGGSPAPAPTPAPAPTPAPAGGGPSGAPLCGGELVDTLQFVCGDRGFYFSRPASRVSARSRGIVEECCFRSCDLALLETYCATPAKSE